European Patent Specification EP 3 774 770 B1, published September 6, 2023. Title: NOVEL HYDRAZONE DERIVATIVES FOR PREVENTING OR TREATING EBV-RELATED CANCERS. Applicant: UNIVERSITE DE BRETAGNE OCCIDENTALE CENTRE HOSPITALIER REGIONAL UNIVERSITAIRE DE BREST INSTITUT NATIONAL DE LA SANTE ET DE LA RECHERCHE MEDICALE CENTRE NATIONAL DE LA RECHERCHE SCIENTIFIQUE INSTITUT CURIE UNIVERSITE PARIS DIDEROT PARIS 7 UNIVERSITE PARIS DESCARTES UNIV PARIS XIII PARIS-NORD VILLETANEUSE UNIV PARIS SUD. The sequence listing filed with the application follows.

SEQUENCE LISTING (3 sequences)

SEQ ID NO: 1 - RNA, 18 nt, Artificial
  Primer
ggggcaggagcaggagga

SEQ ID NO: 2 - RNA, 18 nt, Artificial
  Primer
ggggcaggagcaggagga

SEQ ID NO: 3 - DNA, 26 bp, Artificial
  Primer
caatcggatcgaattcgatccgattg